European Patent Application EP 4 253 434 A1, published October 4, 2023. Title: 基底及其制备方法以及基底的用途. Applicant: 深圳市真迈生物科技有限公司. The sequence listing filed with the application follows.

SEQUENCE LISTING (3 sequences)

SEQ ID NO: 1 - DNA, 26 bp, Artificial Sequence
  misc_feature (1)..(26): 接头序列
tttttttttttttttttttttttttt

SEQ ID NO: 2 - DNA, 27 bp, Artificial Sequence
  misc_feature (1)..(27): 接头序列
caacaacaacaacaacaacaacaacaa

SEQ ID NO: 3 - DNA, 23 bp, Artificial Sequence
  misc_feature (1)..(23): 接头序列
ctgccccgggttcctcattctat